European Patent Application EP 4 640 213 A1, published October 29, 2025. Title: 나트륨 포도당 운반체-2 저해제 및 안지오텐신 Ⅱ 수용체 차단제를 함유하는 경구용 약학 제제. Applicant: 주식회사 티에치팜. The sequence listing filed with the application follows.

SEQUENCE LISTING (4 sequences)

SEQ ID NO: 1 - DNA, 19 bp, synthetic construct
  source 1..19: mol_type = other DNA
caacgccctgctaagcaac

SEQ ID NO: 2 - DNA, 20 bp, synthetic construct
  source 1..20: mol_type = other DNA
actggtgacatcgaggttgg

SEQ ID NO: 3 - DNA, 20 bp, synthetic construct
  source 1..20: mol_type = other DNA
cagtcaacggatttggtcgt

SEQ ID NO: 4 - DNA, 20 bp, synthetic construct
  source 1..20: mol_type = other DNA
ttgattttgcagggatctcg